European Patent Specification EP 3 880 700 B1, published December 17, 2025. Title: Novel c-met and TMX2 Antibodies. Applicant: R.G.C.C. Holdings AG. The sequence listing filed with the application follows.

SEQUENCE LISTING (3 sequences)

SEQ ID NO: 1 - protein, 9 aa, Homo sapiens
VLPEFRDSY

SEQ ID NO: 2 - protein, 9 aa, Homo sapiens
  Designed peptide based on TMX2 AA sequence 86-95 modified by substitution of AA87 (Glu) with Gln
VQQHIGNIF

SEQ ID NO: 3 - protein, 9 aa, Homo sapiens
  Designed peptide based on TMX2 AA sequence 173-181
FAPIYADLS